European Patent Application EP 4 763 865 A1, published June 24, 2026. Title: Anti-c-MET nanobody and use thereof. Applicant: MINGHUI PHARMACEUTICAL (HANGZHOU) LIMITED. Application CN PCT/CN2024/111721, filed August 13, 2024. The sequence listing filed with the application follows.

SEQUENCE LISTING (16 sequences)

SEQ ID NO: 1 - protein, 126 aa, synthetic construct
  source 1..126: note = MHAB07-3 VHH
QLQLVESGGGLVQAGGSLRLSCAASGRITNTYVMGWFRQAPGKERELQAAITWTVGSTYYVDSVKGRFTISRDNAKNTLYLQMNSLKPEDTAVYYCAASRFSAWPPRGTLGEWNSWGQGTQVTVSS

SEQ ID NO: 2 - protein, 5 aa, synthetic construct
  source 1..5: note = MHAB07-3 VHH-CDR1 (Kabat definition)
TYVMG

SEQ ID NO: 3 - protein, 17 aa, synthetic construct
  source 1..17: note = MHAB07-3 VHH-CDR2 (Kabat definition)
AITWTVGSTYYVDSVKG

SEQ ID NO: 4 - protein, 17 aa, synthetic construct
  source 1..17: note = MHAB07-3 VHH-CDR3 (Kabat definition)
SRFSAWPPRGTLGEWNS

SEQ ID NO: 5 - protein, 7 aa, synthetic construct
  source 1..7: note = MHAB07-3 VHH-CDR1 (Chothia definition)
GRITNTY

SEQ ID NO: 6 - protein, 6 aa, synthetic construct
  source 1..6: note = MHAB07-3 VHH-CDR2 (Chothia definition)
TWTVGS

SEQ ID NO: 7 - protein, 17 aa, synthetic construct
  source 1..17: note = MHAB07-3 VHH-CDR3 (Chothia definition)
SRFSAWPPRGTLGEWNS

SEQ ID NO: 8 - protein, 8 aa, synthetic construct
  source 1..8: note = MHAB07-3 VHH-CDR1 (IMGT definition)
GRITNTYV

SEQ ID NO: 9 - protein, 8 aa, synthetic construct
  source 1..8: note = MHAB07-3 VHH-CDR2 (IMGT definition)
ITWTVGST

SEQ ID NO: 10 - protein, 19 aa, synthetic construct
  source 1..19: note = MHAB07-3 VHH-CDR3 (IMGT definition)
AASRFSAWPPRGTLGEWNS

SEQ ID NO: 11 - protein, 358 aa, synthetic construct
  source 1..358: note = MHAB07-3
QLQLVESGGGLVQAGGSLRLSCAASGRITNTYVMGWFRQAPGKERELQAAITWTVGSTYYVDSVKGRFTISRDNAKNTLYLQMNSLKPEDTAVYYCAASRFSAWPPRGTLGEWNSWGQGTQVTVSSEPKSSDKTHTCPPCPAPEAAGGPSVFLFPPKPKDTLMISRTPEVTCVVVDVSHEDPEVKFNWYVDGVEVHNAKTKPREEQYNSTYRVVSVLTVLHQDWLNGKEYKCKVSNKALPAPIEKTISKAKGQPREPQVYTLPPSREEMTKNQVSLTCLVKGFYPSDIAVEWESNGQPENNYKTTPPVLDSDGSFFLYSKLTVDKSRWQQGNVFSCSVMHEALHNHYTQKSLSLSPGK

SEQ ID NO: 12 - protein, 358 aa, synthetic construct
  source 1..358: note = MHAB07-3-1
QLQLVESGGGLVQPGGSLRLSCAASGRITNTYVMGWVRQAPGKEREFQAAITWTVGSTYYVDSVKGRFTISRDNAKNTLYLQMNSLRPEDTAVYYCAASRFSAWPPRGTLGEWNSWGQGTQVTVSSEPKSSDKTHTCPPCPAPEAAGGPSVFLFPPKPKDTLMISRTPEVTCVVVDVSHEDPEVKFNWYVDGVEVHNAKTKPREEQYNSTYRVVSVLTVLHQDWLNGKEYKCKVSNKALPAPIEKTISKAKGQPREPQVYTLPPSREEMTKNQVSLTCLVKGFYPSDIAVEWESNGQPENNYKTTPPVLDSDGSFFLYSKLTVDKSRWQQGNVFSCSVMHEALHNHYTQKSLSLSPGK

SEQ ID NO: 13 - protein, 358 aa, synthetic construct
  source 1..358: note = MHAB07-3-2
QLQLVESGGGLVQPGGSLRLSCAASGRITNTYVMGWVRQAPGKEREFVAAITWTVGSTYYVDSVKGRFTISRDNAKNTLYLQMNSLRPEDTAVYYCAASRFSAWPPRGTLGEWNSWGQGTQVTVSSEPKSSDKTHTCPPCPAPEAAGGPSVFLFPPKPKDTLMISRTPEVTCVVVDVSHEDPEVKFNWYVDGVEVHNAKTKPREEQYNSTYRVVSVLTVLHQDWLNGKEYKCKVSNKALPAPIEKTISKAKGQPREPQVYTLPPSREEMTKNQVSLTCLVKGFYPSDIAVEWESNGQPENNYKTTPPVLDSDGSFFLYSKLTVDKSRWQQGNVFSCSVMHEALHNHYTQKSLSLSPGK

SEQ ID NO: 14 - protein, 126 aa, synthetic construct
  source 1..126: note = MHAB07-3-1 VHH
QLQLVESGGGLVQPGGSLRLSCAASGRITNTYVMGWVRQAPGKEREFQAAITWTVGSTYYVDSVKGRFTISRDNAKNTLYLQMNSLRPEDTAVYYCAASRFSAWPPRGTLGEWNSWGQGTQVTVSS

SEQ ID NO: 15 - protein, 126 aa, synthetic construct
  source 1..126: note = MHAB07-3-2 VHH
QLQLVESGGGLVQPGGSLRLSCAASGRITNTYVMGWVRQAPGKEREFVAAITWTVGSTYYVDSVKGRFTISRDNAKNTLYLQMNSLRPEDTAVYYCAASRFSAWPPRGTLGEWNSWGQGTQVTVSS

SEQ ID NO: 16 - protein, 232 aa, synthetic construct
  source 1..232: note = Fc (LALA) of human IgG1
EPKSSDKTHTCPPCPAPEAAGGPSVFLFPPKPKDTLMISRTPEVTCVVVDVSHEDPEVKFNWYVDGVEVHNAKTKPREEQYNSTYRVVSVLTVLHQDWLNGKEYKCKVSNKALPAPIEKTISKAKGQPREPQVYTLPPSREEMTKNQVSLTCLVKGFYPSDIAVEWESNGQPENNYKTTPPVLDSDGSFFLYSKLTVDKSRWQQGNVFSCSVMHEALHNHYTQKSLSLSPGK